European Patent Application EP 4 446 344 A1, published October 16, 2024. Title: ANTI-CD24 ANTIBODY AND USE THEREOF. Applicant: Beijing Kanghong Biomedical Co., Ltd. The sequence listing filed with the application follows.

SEQUENCE LISTING (157 sequences)

SEQ ID NO: 1 - protein, 6 aa, synthetic construct
RGYSWH

SEQ ID NO: 2 - protein, 6 aa, synthetic construct
NGYSWH

SEQ ID NO: 3 - protein, 6 aa, synthetic construct
SGYTWH

SEQ ID NO: 4 - protein, 6 aa, synthetic construct
RGYTWH

SEQ ID NO: 5 - protein, 5 aa, synthetic construct
TYGVS

SEQ ID NO: 6 - protein, 16 aa, synthetic construct
YIHHRGSTNYNPSLKS

SEQ ID NO: 7 - protein, 16 aa, synthetic construct
YIHHRGTTNYNPSLKS

SEQ ID NO: 8 - protein, 16 aa, synthetic construct
YIHHSGSTNYNPSLKS

SEQ ID NO: 9 - protein, 16 aa, synthetic construct
VIWGDGSTNYHSALIS

SEQ ID NO: 10 - protein, 16 aa, synthetic construct
YIHYSGNTNYNPSLKS

SEQ ID NO: 11 - protein, 16 aa, synthetic construct
YIQFSGSTKYNPSLKS

SEQ ID NO: 12 - protein, 16 aa, synthetic construct
YIQYSGSTNYNPSLKS

SEQ ID NO: 13 - protein, 16 aa, synthetic construct
FIHYSGTTNYNPSLKS

SEQ ID NO: 14 - protein, 16 aa, synthetic construct
YIHHRGTTNYNPSLKN

SEQ ID NO: 15 - protein, 16 aa, synthetic construct
YIHHSGATNYNPSLKS

SEQ ID NO: 16 - protein, 16 aa, synthetic construct
YIHYSGSTKYNPSLKS

SEQ ID NO: 17 - protein, 16 aa, synthetic construct
YIHYSGSTNYNPSLKS

SEQ ID NO: 18 - protein, 16 aa, synthetic construct
YTQYSGSTNYNPSLKS

SEQ ID NO: 19 - protein, 8 aa, synthetic construct
GTNSAFDY

SEQ ID NO: 20 - protein, 8 aa, synthetic construct
GTDRSFDY

SEQ ID NO: 21 - protein, 8 aa, synthetic construct
GSTWAFDH

SEQ ID NO: 22 - protein, 8 aa, synthetic construct
GTTGGLDY

SEQ ID NO: 23 - protein, 8 aa, synthetic construct
GTTTALDY

SEQ ID NO: 24 - protein, 8 aa, synthetic construct
GSDRAFDY

SEQ ID NO: 25 - protein, 9 aa, synthetic construct
YYGYDFFAY

SEQ ID NO: 26 - protein, 9 aa, synthetic construct
YYGYDFFPY

SEQ ID NO: 27 - protein, 17 aa, synthetic construct
KSSQSLLYSNNQKNYLA

SEQ ID NO: 28 - protein, 17 aa, synthetic construct
KSSQSLLYSSDQKNYLA

SEQ ID NO: 29 - protein, 17 aa, synthetic construct
KSSQSLLYSKNQKNYSA

SEQ ID NO: 30 - protein, 17 aa, synthetic construct
KSSQSLLYSNNQKNYLT

SEQ ID NO: 31 - protein, 17 aa, synthetic construct
KSSQSLLYSSDQKNYLT

SEQ ID NO: 32 - protein, 17 aa, synthetic construct
KSSQSLLYSSNQKNYLA

SEQ ID NO: 33 - protein, 17 aa, synthetic construct
QSSQSLLYSSNQKNYLV

SEQ ID NO: 34 - protein, 17 aa, synthetic construct
QSSQSLLYSNNQKNYLV

SEQ ID NO: 35 - protein, 11 aa, synthetic construct
RASQDISNYLN

SEQ ID NO: 36 - protein, 10 aa, synthetic construct
SASSSISYMH

SEQ ID NO: 37 - protein, 10 aa, synthetic construct
SASSSLSYMH

SEQ ID NO: 38 - protein, 12 aa, synthetic construct
SASSSVSSSYLY

SEQ ID NO: 39 - protein, 10 aa, synthetic construct
SASSSVSYMH

SEQ ID NO: 40 - protein, 7 aa, synthetic construct
WASTRES

SEQ ID NO: 41 - protein, 7 aa, synthetic construct
WASTKAS

SEQ ID NO: 42 - protein, 7 aa, synthetic construct
DTSKLAS

SEQ ID NO: 43 - protein, 7 aa, synthetic construct
LASTRES

SEQ ID NO: 44 - protein, 7 aa, synthetic construct
STSNLAS

SEQ ID NO: 45 - protein, 7 aa, synthetic construct
WASTRAS

SEQ ID NO: 46 - protein, 7 aa, synthetic construct
WASTRYS

SEQ ID NO: 47 - protein, 7 aa, synthetic construct
YTSRLHS

SEQ ID NO: 48 - protein, 9 aa, synthetic construct
QQYYIYPLT

SEQ ID NO: 49 - protein, 9 aa, synthetic construct
QQYYIYPFT

SEQ ID NO: 50 - protein, 9 aa, synthetic construct
FQGSGYPLT

SEQ ID NO: 51 - protein, 9 aa, synthetic construct
HQRSSYPCT

SEQ ID NO: 52 - protein, 9 aa, synthetic construct
HQWSSYPPT

SEQ ID NO: 53 - protein, 9 aa, synthetic construct
QQGNTLPHT

SEQ ID NO: 54 - protein, 9 aa, synthetic construct
QQYFIYPFT

SEQ ID NO: 55 - protein, 9 aa, synthetic construct
QQYFIYPMS

SEQ ID NO: 56 - protein, 9 aa, synthetic construct
QQYFLYPMS

SEQ ID NO: 57 - protein, 117 aa, synthetic construct
DVQLQESGPDLVKPSQSLSLTCTVTGHSITRGYSWHWIRQFPGNKLEWMGYIHHRGTTNYNPSLKSRISFTRDTSKNQFFLQLNSLTTEDTATYFCSRGTNSAFDYWGQGTTLTVSS

SEQ ID NO: 58 - protein, 117 aa, synthetic construct
DVQLQESGPDLVKPSHSLSLTCTVTGYSITRGYSWHWIRQFPGNKLEWMGYIHYSGSTNYNPSLKSRISFTRDTSKNQFFLNLTSLTSEDTATYYCSRGSTWAFDHWGQGTILTVSS

SEQ ID NO: 59 - protein, 117 aa, synthetic construct
DVQLQESGPDLVKPSQSLSLTCTVTGHSITRGYSWHWIRQFPGNKLEWMGYIHHRGSTNYNPSLKSRISFTRDTSKNQFFLQLNSLTTEDTATYFCSRGTNSAFDYWGQGTTLTVSS

SEQ ID NO: 60 - protein, 117 aa, synthetic construct
DVQLQESGPDLVKPSQSLSLTCTVTGHSITRGYSWHWIRQFPGNKLEWMGYIHHRGSTNYNPSLKSRISFTRDTSKNQFFLQLNSLTTEDTATYFCLRGTNSAFDYWGQGTTLTVSS

SEQ ID NO: 61 - protein, 117 aa, synthetic construct
DVQLQESGPDLVKPSQSLSLTCTVTGHSITNGYSWHWIRQFPGNKLEWMGYIHHSGSTNYNPSLKSRISFTRDTSKNQFFLQLNSLTTEDTATYYCLRGTDRSFDYWGQGTTLTVSS

SEQ ID NO: 62 - protein, 117 aa, synthetic construct
DVQLQESGPDLVNPSQSLSLTCTVTGYSISRGYSWHWLRRFPGNKLEWMGFIHYSGTTNYNPSLKSRISFTRDTSKNQFFLQLNSLTTEDTATYYCLRGTDRSFDYWGQGTTLTVSS

SEQ ID NO: 63 - protein, 117 aa, synthetic construct
DVQLQESGPDLEKPSQSLSLTCTVTGYSITRGYSWHWIRQFPGNKLEWMGYIHYSGSTKYNPSLKSRVSFTRDTSKNQFFLQLNSLSPEDTATYYCSRGSDRAFDYWGQGTTLTVSS

SEQ ID NO: 64 - protein, 117 aa, synthetic construct
QVQLKESGPGLVAPSQSLSITCTVSGFSLTTYGVSWVRQPPGKGLEWLGVIWGDGSTNYHSALISRLTISKDNSKSQVFLKLNSLQTDDTATYYCAFYYGYDFFAYWGQGTLVTVSA

SEQ ID NO: 65 - protein, 117 aa, synthetic construct
QVQLKESGPGLVTPSQSLSITCTVSGFSLTTYGVSWVRQPPGKGLEWLGVIWGDGSTNYHSALISRLSISKDNSKSQVFLKLNSLQTDDTATYYCAFYYGYDFFPYWGQGTLVTVSA

SEQ ID NO: 66 - protein, 117 aa, synthetic construct
DVQLQESGPDLVKPSHSFSLTCTVTGYSITRGYSWHWIRQFPGNKLEWMGYIHYSGNTNYNPSLKSRFSFTRDTSKNQFFLNLTSLTSEDTATYYCSRGSTWAFDHWGQGTILTVSS

SEQ ID NO: 67 - protein, 117 aa, synthetic construct
DVQLQESGPDLVKPSQSLSLTCTVTGYSITSGYTWHWIRQFPGNKLEWMGYIQYSGSTNYNPSLKSRISFTRDTSKNQFFLQLNSVTTEDTATYYCARGTTGGLDYWGQGTTLTVSS

SEQ ID NO: 68 - protein, 117 aa, synthetic construct
DVQLQESGPDLVKPSQSLSLTCTVTGYSITSGYTWHWIRQFPGNKLEWMGYTQYSGSTNYNPSLKSRISFTRDTSKNQFFLQLNSVTTEDTATYYCARGTTGGLDYWGQGTTLTVSS

SEQ ID NO: 69 - protein, 117 aa, synthetic construct
DVQLQESGPDLVKPSQSLSLTCTVTGHSITSGYTWHWIRQFPGNKLEWMGYIHHSGATNYNPSLKSRISFTRDTSKNQFFLQLNSLTTEDTATYYCLRGTDRSFDYWGQGTTLTVSS

SEQ ID NO: 70 - protein, 117 aa, synthetic construct
DVQLQESGPDLVKPSQSLSLTCTVTGYSITRGYTWHWIRQFPGNKLEWMGYIQFSGSTKYNPSLKSRFSITRDTSKNQFFLQLNSVTTEDTATYYCARGTTTALDYWGQGTSVTVSS

SEQ ID NO: 71 - protein, 117 aa, synthetic construct
DVQLQESGPDLVKPSQSLSLTCTVTGHSITRGYSWHWIRQFPGNKLEWMGYIHHRGTTNYNPSLKNRISFTRDTSKNQFFLQLNSLTTEDTATYFCSRGTNSAFDYWGQGTTLTVSS

SEQ ID NO: 72 - protein, 107 aa, synthetic construct
DIQMTQTTSSLSASLGDRVTISCRASQDISNYLNWYQQKPDGTVKLLIYYTSRLHSGVPSRFSGSGSGTDYSLTISNLEQEDIATYFCQQGNTLPHTFGGGTKLEIK

SEQ ID NO: 73 - protein, 113 aa, synthetic construct
DIVMSQSPSSLAVSVGEKITMSCKSSQSLLYSNNQKNYLAWYQQIPGQSPKLLIYLASTRESGVPDRFTGSGSGTDFTLTISSVKAEDLAVYYCQQYFIYPMSFGSGTKLEIK

SEQ ID NO: 74 - protein, 113 aa, synthetic construct
DIVMSQSPSSLTVSVGEKITMSCKSSQSLLYSSDQKNYLAWYQQNPGQSPKLLIYWASTRASGVPDRFTGSGSGTDFTLTISSVKAEDLAIYYCQQYYIYPLTFGSGTKLEIK

SEQ ID NO: 75 - protein, 113 aa, synthetic construct
DIVMSQSPSSLTVSVGEKITMSCKSSQSLLYSSDQKNYLAWYQQNPGQSPKLLIYWASTKASGVPDRFTGSGSGTDFTLTISSVKAEDLAVYYCQQYYIYPLTFGSGTKLEIK

SEQ ID NO: 76 - protein, 113 aa, synthetic construct
DIVMSQSPSSLVVSVGEKISMSCKSSQSLLYSNNQKNYLAWYQQIPGQSPKLLIYWASTRESGVPDRFTGSGSGTDFTLTISSVKAEDLAVYYCQQYYIYPLTFGSGTKLEIK

SEQ ID NO: 77 - protein, 113 aa, synthetic construct
DIVMSQSPSSLAVSIGEKVTMNCQSSQSLLYSNNQKNYLVWYQQKPGQSPKLLIHWASTRESGVPDRFTGSGSGTDFTLTISSVKAEDLAVYYCQQYYIYPFTFGSGTKLEIK

SEQ ID NO: 78 - protein, 106 aa, synthetic construct
ENVLTQSPAIMSASPGEKVTMTCSASSSLSYMHWYQQKSSTSPKVWIYDTSKLASGVPGRFSGSGSGNSYSLTISSMEAEDVATYYCFQGSGYPLTFGAGTKLEVK

SEQ ID NO: 79 - protein, 106 aa, synthetic construct
ENVLTQSPAIMSTSPGEKVTMTCSASSSVSYMHWYQQKSNTSPKVWIYDTSKLASGVPGRFSGSGSGNSYSLTISSMEAEDVATYYCFQGSGYPLTFGAGTKLEVK

SEQ ID NO: 80 - protein, 113 aa, synthetic construct
DIVMSQSPSSLTVSVGEKVTMSCKSSQSLLYSSNQKNYLAWYQQKPGQSPKLLIYWASTRESGVPDRFTGSGSGTDFTLTISSVKAEDLAVYYCQQYYIYPLTFGAGTKLELK

SEQ ID NO: 81 - protein, 113 aa, synthetic construct
DIVMSQSPSSLTVSVGEKITMSCKSSQSLLYSSDQKNYLAWYQQIPGQSPKLLIYWASTKASGVPDRFTGSGSGTDFTLTISSVKAEDLAVYYCQQYYIYPLTFGSGTKLEIK

SEQ ID NO: 82 - protein, 113 aa, synthetic construct
DIVMSQSPSSLTVSVGEKVTMSCKSSQSLLYSSDQKNYLTWYQQKPGQSPKLLIYWASTRYSGVPDRFTGSGSGTDFTLTISSVKAEDLAVYYCQQYYIYPFTFGSGTKLEIK

SEQ ID NO: 83 - protein, 113 aa, synthetic construct
DIVMSQSPSSLAVSVGEKITMNCKSSQSLLYSNNQKNYLAWYQQIPGQSPKLLIYLASTRESGVPDRFTGSGSGTDFTLTISSVKAEDLAVYYCQQYFLYPMSFGSGTKLEIK

SEQ ID NO: 84 - protein, 113 aa, synthetic construct
DIVMSQSPSSLAVSVGENITMTCKSSQSLLYSNNQKNYLTWYQQNPGQSPKLLIYWASTRESGVPDRFTGSGSGTDFTLTISSVKAEDLAVYYCQQYYIYPFTFGSGTKLEIK

SEQ ID NO: 85 - protein, 113 aa, synthetic construct
GIVMSQSPSSLAVSVGENITMTCKSSQSLLYSNNQKNYLTWYQQNPGQSPKLLIYWASTRESGVPDRFTGSGSGTDFTLTISSVKAEDLAVYYCQQYYIYPFTFGSGTKLEIK

SEQ ID NO: 86 - protein, 113 aa, synthetic construct; identical to SEQ ID NO: 75

SEQ ID NO: 87 - protein, 113 aa, synthetic construct; identical to SEQ ID NO: 75

SEQ ID NO: 88 - protein, 113 aa, synthetic construct; identical to SEQ ID NO: 75

SEQ ID NO: 89 - protein, 113 aa, synthetic construct
DIVMSQSPSSLAVSVGEKVTVSCKSSQSLLYSSDQKNYLTWYQQKPGQSPKLLIYWASTRESGVPDRFTGGGSGTDFTLTISSVRAEDLAVYYCQQYFIYPFTFGSGTKLEIK

SEQ ID NO: 90 - protein, 113 aa, synthetic construct; identical to SEQ ID NO: 75

SEQ ID NO: 91 - protein, 113 aa, synthetic construct
DIVMSQSPSSLAVSIGEKVTMNCQSSQSLLYSSNQKNYLVWYQQKPGQSPKLLIHWASTRESGVPDRFTGSGSGTDFTLTISSVKAEDLAVYYCQQYYIYPFTFGSGTKLEIK

SEQ ID NO: 92 - protein, 113 aa, synthetic construct
DIVMSQSPSSLAVSVGEKVTLNCKSSQSLLYSKNQKNYSAWYQQKPGQSPKLLIYWASTRESGVPDRFTGSGSGTDFTLTISSVKAEDLAVYYCQQYYIYPLTFGAGTKLELK

SEQ ID NO: 93 - protein, 108 aa, synthetic construct
QIVLTQSPAIMSASPGEKVTLTCSASSSVSSSYLYWYQQKPGSSPKLWIYSTSNLASGVPARFSGSGSGTSYSLTISSMEAEDAASYFCHQWSSYPPTFGAGTKLELK

SEQ ID NO: 94 - protein, 106 aa, synthetic construct
QIVLTQSPAIMSASPGEKVTMTCSASSSISYMHWYQQKPGTSPKRWIYDTSKLASGVPARFSGSGSGTSYSLTISSMEAEDAATYYCHQRSSYPCTFGGGTKLEIK

SEQ ID NO: 95 - protein, 330 aa, synthetic construct
AKTTAPSVYPLAPVCGDTTGSSVTLGCLVKGYFPEPVTLTWNSGSLSSGVHTFPAVLQSDLYTLSSSVTVTSSTWPSQSITCNVAHPASSTKVDKKIEPRGPTIKPCPPCKCPAPNLLGGPSVFIFPPKIKDVLMISLSPIVTCVVVDVSEDDPDVQISWFVNNVEVHTAQTQTHREDYNSTLRVVSALPIQHQDWMSGKEFKCKVNNKDLPAPIERTISKPKGSVRAPQVYVLPPPEEEMTKKQVTLTCMVTDFMPEDIYVEWTNNGKTELNYKNTEPVLDSDGSYFMYSKLRVEKKNWVERNSYSCSVVHEGLHNHHTTKSFSRTPGK

SEQ ID NO: 96 - protein, 336 aa, synthetic construct
AKTTPPSVYPLAPGCGDTTGSSVTLGCLVKGYFPESVTVTWNSGSLSSSVHTFPALLQSGLYTMSSSVTVPSSTWPSQTVTCSVAHPASSTTVDKKLEPSGPISTINPCPPCKECHKCPAPNLEGGPSVFIFPPNIKDVLMISLTPKVTCVVVDVSEDDPDVQISWFVNNVEVHTAQTQTHREDYNSTIRVVSTLPIQHQDWMSGKEFKCKVNNKDLPSPIERTISKIKGLVRAPQVYILPPPAEQLSRKDVSLTCLVVGFNPGDISVEWTSNGHTEENYKDTAPVLDSDGSYFIYSKLNMKTSKWEKTDSFSCNVRHEGLKNYYLKKTISRSPGK

SEQ ID NO: 97 - protein, 107 aa, synthetic construct
RADAAPTVSIFPPSSEQLTSGGASVVCFLNNFYPKDINVKWKIDGSERQNGVLNSWTDQDSKDSTYSMSSTLTLTKDEYERHNSYTCEATHKTSTSPIVKSFNRNEC

SEQ ID NO: 98 - protein, 117 aa, synthetic construct
QVQLQESGPGLVKPSQTLSLTCTVSGHSITRGYSWHWIRQHPGKGLEWIGYIHHRGSTNYNPSLKSRVTISVDTSKNQFSLKLSSVTAADTAVYYCARGTNSAFDYWGQGTLVTVSS

SEQ ID NO: 99 - protein, 117 aa, synthetic construct
QVQLQESGPGLVKPSQTLSLTCTVSGHSITRGYSWHWIRQHPGNGLEWIGYIHHRGSTNYNPSLKSRVTISRDTSKNQFSLKLSSVTAADTAVYYCARGTNSAFDYWGQGTLVTVSS

SEQ ID NO: 100 - protein, 117 aa, synthetic construct
QVQLQESGPGLVKPSETLSLTCTVTGGSISRGYSWHWVRQAPGQRLEWMGYIHHRGSTNYNPSLKSRITINPDTSKNQFSLQLNSVTPEDTAVYYCARGTNSAFDYWGQGTLVTVSS

SEQ ID NO: 101 - protein, 117 aa, synthetic construct
QVQLQESGPGLVKPSQTLSLTCTVSGHSITRGYSWHWIRQHPGNGLEWIGYIHHRGSTNYNPSLKSRVTISVDTSKNQFSLKLSSVTAADTAVYYCARGTNSAFDYWGQGTLVTVSS

SEQ ID NO: 102 - protein, 117 aa, synthetic construct
QVQLQESGPGLVKPSQTLSLTCTVSGGSISRGYSWHWVRQAPGQRLEWMGYIHHRGSTNYNPSLKSRITINPDTSKNQFSLQLNSVTPEDTAVYYCARGTNSAFDYWGQGTLVTVSS

SEQ ID NO: 103 - protein, 117 aa, synthetic construct
QVQLQESGPGLVKPSQTLSLTCTVSGHSITNGYSWHWIRQHPGNGLEWMGYIHHSGSTNYNPSLKSRVTISVDTSKNQFSLKLSSVTAADTAVYYCARGTDRSFDYWGQGTLVTVSS

SEQ ID NO: 104 - protein, 117 aa, synthetic construct
QVQLQESGPGLVKPSETLSLTCTVSGYSISRGYSWHWVRQMPGKELEWMGYIHYSGNTNYNPSLKSRITINPDTSKNQFSLQLNSVTPEDTAVYYCARGSTWAFDHWGQGTLVTVSS

SEQ ID NO: 105 - protein, 117 aa, synthetic construct
QVQLQESGPGLVKPSETLSLTCTVSGYSITRGYSWHWIRQPPGNGLEWMGYIHYSGNTNYNPSLKSRVTISVDTSKNQFSLKLSSVTAADTAVYYCARGSTWAFDHWGQGTMVTVSS

SEQ ID NO: 106 - protein, 117 aa, synthetic construct
QVQLQESGPGLVKPSQTLSLTCTVSGHSITNGYSWHWIRQHPGNGLEWIGYIHHSGSTNYNPSLKSRVTISVDTSKNQFSLKLSSVTAADTAVYYCARGTDRSFDYWGQGTLVTVSS

SEQ ID NO: 107 - protein, 117 aa, synthetic construct
QVQLQESGPGLVKPSQTLSLTCTVSGHSITNGYSWHWIRQHPGNGLEWMGYIHHSGSTNYNPSLKSRVTISRDTSKNQFSLKLSSVTAADTAVYYCARGTDRSFDYWGQGTLVTVSS

SEQ ID NO: 108 - protein, 117 aa, synthetic construct
QVQLQESGPGLVKPSETLSLTCTVSGYSISRGYSWHWVRQMPGKELEWMGYIHYSGNTNYNPSLKSRITMSVDTSKNQFYLKLSSVTAADTAVYYCARGSTWAFDHWGQGTLVTVSS

SEQ ID NO: 109 - protein, 117 aa, synthetic construct
QVQLQESGPGLVKPSETLSLTCTVSGYSITRGYSWHWIRQPPGNGLEWIGYIHYSGNTNYNPSLKSRVTISVDTSKNQFSLKLSSVTAADTAVYYCARGSTWAFDHWGQGTMVTVSS

SEQ ID NO: 110 - protein, 117 aa, synthetic construct
QVQLQESGPGLVKPSETLSLTCTVSGYSITRGYSWHWIRQPPGNGLEWMGYIHYSGNTNYNPSLKSRVTISRDTSKNQFSLKLSSVTAADTAVYYCARGSTWAFDHWGQGTMVTVSS

SEQ ID NO: 111 - protein, 117 aa, synthetic construct
QVQLQESGPGLVKPSETLSLTCTVSGYSISRGYSWHWIRQPPGKGLEWIGYIHHRGSTNYNPSLKSRVTISVDTSKNQFSLKLSSVTAADTAVYYCARGTNSAFDYWGQGTLVTVSS

SEQ ID NO: 112 - protein, 117 aa, synthetic construct
QVQLQESGPGLVKPSETLSLTCTVTGGSISNGYSWHWVRQMPGKGLEWMGYIHHSGSTNYNPSLKSRITINPDTSKNQFSLQLNSVTPEDTAVYYCARGTDRSFDYWGQGTLVTVSS

SEQ ID NO: 113 - protein, 117 aa, synthetic construct
QVQLQESGPGLVKPSETLSLTCTVSGYSITRGYSWHWIRQPPGKGLEWIGYIHYSGNTNYNPSLKSRVTISVDTSKNQFSLKLSSVTAADTAVYYCARGSTWAFDHWGQGTMVTVSS

SEQ ID NO: 114 - protein, 117 aa, synthetic construct
QVQLQESGPELVKPSQTLSLTCTVSGHSITRGYSWHWIRQFPGRKLEWMGYIHHRGSTNYNPSLKSRLTISRDTSKNQFYLQLRSVTSDDTAVYYCSRGTNSAFDYWGQGTLVTVSS

SEQ ID NO: 115 - protein, 117 aa, synthetic construct; identical to SEQ ID NO: 101

SEQ ID NO: 116 - protein, 117 aa, synthetic construct
QVQLQESGPELVKPSQTLSLTCTVSGHSITRGYSWHWIRQFPGRKLEWMGYIHHRGSTNYNPSLKSRLTISRDTSKNQFYLQLRSVTSDDTAVYYCARGTNSAFDYWGQGTLVTVSS

SEQ ID NO: 117 - protein, 117 aa, synthetic construct
QVQLQESGPGLVKPSQSLSLTCTVSGHSITRGYSWHWIRQHPGKGLEWIGYIHHRGSTNYNPSLKSRVTISRDTSKNQFSLQLNSLTAEDTAVYYCARGTNSAFDYWGQGTLVTVSS

SEQ ID NO: 118 - protein, 117 aa, synthetic construct
QVQLQESGPGLVKPSQSLSLTCTVSGHSITRGYSWHWIRQAPGKGLEWVGYIHHRGSTNYNPSLKSRFTISRDTSKNQFYLQLNSLTAEDTAVYYCARGTNSAFDYWGQGTLVTVSS

SEQ ID NO: 119 - protein, 117 aa, synthetic construct
QVQLQESGPGLVKPSETLSLTCTVTGGSISNGYSWHWVRQAPGQRLEWMGYIHHSGSTNYNPSLKSRITINPDTSKNQFSLQLNSVTPEDTAVYYCARGTDRSFDYWGQGTLVTVSS

SEQ ID NO: 120 - protein, 117 aa, synthetic construct
QVQLQESGPGLVKPSQTLSLTCTVSGHSITNGYSWHWIRQHPGKGLEWIGYIHHSGSTNYNPSLKSRVTISVDTSKNQFSLKLSSVTAADTAVYYCARGTDRSFDYWGQGTLVTVSS

SEQ ID NO: 121 - protein, 113 aa, synthetic construct
DIVMTQSPDSLAVSLGERATINCKSSQSLLYSSNQKNYLAWYQQKPGQPPKLLIYWASTRESGVPDRFSGSGSGTDFTLTISSLQAEDVAVYYCQQYYIYPLTFGGGTKVEIK

SEQ ID NO: 122 - protein, 113 aa, synthetic construct
DIVMTQSPDSLAVSLGERATISCKSSQSLLYSSNQKNYLAWYQQKPGQSPKLLIYWASTRESGVPDRFTGSGSGTDFTLTISSLQAEDVAVYYCQQYYIYPLTFGGGTKVEIK

SEQ ID NO: 123 - protein, 113 aa, synthetic construct
DIVMTQSPDSLAVSLGERATISCKSSQSLLYSSDQKNYLTWYQQKPGQSPKLLIYWASTRYSGVPDRFSGSGSGTDFTLTISSLQAEDVAVYYCQQYYIYPFTFGQGTKLEIK

SEQ ID NO: 124 - protein, 113 aa, synthetic construct
DIVMTQSPDSLAVSLGERATISCKSSQSLLYSSDQKNYLAWYQQKPGQSPKLLIYWASTRASGVPDRFSGSGSGTDFTLTISSLQAEDVAVYYCQQYYIYPLTFGGGTKVEIK

SEQ ID NO: 125 - protein, 113 aa, synthetic construct
DIVMTQSPDSLAVSLGERATINCKSSQSLLYSSDQKNYLTWYQQKPGQPPKLLIYWASTRYSGVPDRFSGSGSGTDFTLKISRVEAEDVGVYYCQQYYIYPFTFGQGTKLEIK

SEQ ID NO: 126 - protein, 113 aa, synthetic construct
DIVMTQSPDSLAVSLGERATISCKSSQSLLYSSDQKNYLTWYQQKPGQPPKLLIYWASTRYSGVPDRFSGSGSGTDFTLTISSLQAEDVAVYYCQQYYIYPFTFGQGTKLEIK

SEQ ID NO: 127 - protein, 113 aa, synthetic construct
DIVMTQSPDSLAVSLGERATINCKSSQSLLYSSNQKNYLAWYQQKPGQAPRLLIYWASTRESGIPDRFSGSGSGTDFTLTISRLEPEDFAVYYCQQYYIYPLTFGQGTKLEIK

SEQ ID NO: 128 - protein, 113 aa, synthetic construct
DIVMTQSPDSLAVSLGERATISCKSSQSLLYSSDQKNYLTWYQQKPGQPPKLLIYWASTRESGVPDRFSGSGSGTDFTLTISSLQAEDVAVYYCQQYFIYPFTFGQGTKLEIK

SEQ ID NO: 129 - protein, 113 aa, synthetic construct
DIVMTQSPDSLAVSLGERATISCKSSQSLLYSSDQKNYLTWYQQKPGQSPKLLIYWASTRESGVPDRFSGGGSGTDFTLTISSLQAEDVAVYYCQQYFIYPFTFGQGTKLEIK

SEQ ID NO: 130 - protein, 113 aa, synthetic construct
DIVMTQSPDSLAVSLGERATINCKSSQSLLYSSDQKNYLTWYQQKPGQPPKLLIYWASTRYSGIPDRFSGSGSGTDFTLTISRLEPEDFAVYYCQQYYIYPFTFGQGTKLEIK

SEQ ID NO: 131 - protein, 113 aa, synthetic construct
DIQMTQSPSSLSASVGDRVTITCKSSQSLLYSSDQKNYLAWYQQKPGQPPKLLIYWASTRASGVPDRFSGSGSGTDFTLTISSLQAEDVAVYYCQQYYIYPLTFGGGTKVEIK

SEQ ID NO: 132 - protein, 113 aa, synthetic construct
DIQMTQSPSSLSASVGDRVTITCKSSQSLLYSSDQKNYLAWYQQKPGQPPKLLIYWASTRASGVPDRFSGSGSGTDFTLKISRVEAEDVGVYYCQQYYIYPLTFGGGTKVEIK

SEQ ID NO: 133 - protein, 113 aa, synthetic construct
DIVMTQSPDSLAVSLGERATISCKSSQSLLYSSDQKNYLAWYQQKPGQPPKLLIYWASTRASGVPDRFSGSGSGTDFTLTISSLQAEDVAVYYCQQYYIYPLTFGGGTKVEIK

SEQ ID NO: 134 - protein, 113 aa, synthetic construct
DIVMTQSPDSLAVSLGERATISCKSSQSLLYSSDQKNYLAWYQQKPGQSPKLLIYWASTRASGVPDRFTGSGSGTDFTLTISSLQAEDVAVYYCQQYYIYPLTFGGGTKVEIK

SEQ ID NO: 135 - protein, 113 aa, synthetic construct
DIVMTQSPDSLAVSLGERATINCKSSQSLLYSSNQKNYLAWYQQKPGQAPRLLIYWASTRESGVPDRFSGSGSGTDFTLTISSLQAEDVAVYYCQQYYIYPLTFGQGTKLEIK

SEQ ID NO: 136 - protein, 113 aa, synthetic construct
DIQMTQSPSSLSASVGDRVTITCKSSQSLLYSSNQKNYLAWFQQKPGKAPKSLIYWASTRESGVPSRFSGSGSGTDFTLTISSLQPEDFATYYCQQYYIYPLTFGQGTKVEIK

SEQ ID NO: 137 - protein, 113 aa, synthetic construct
DIVMTQSPDSLAVSLGERATISCKSSQSLLYSSNQKNYLAWYQQKPGQPPKLLIYWASTRESGVPDRFSGSGSGTDFTLTISSLQAEDVAVYYCQQYYIYPLTFGGGTKVEIK

SEQ ID NO: 138 - protein, 113 aa, synthetic construct
DIVMTQSPDSLAVSLGERATINCKSSQSLLYSSDQKNYLTWYQQKPGQPPKLLIYWASTRESGIPDRFSGSGSGTDFTLTISRLEPEDFAVYYCQQYFIYPFTFGQGTKLEIK

SEQ ID NO: 139 - protein, 113 aa, synthetic construct
DIVMTQSPDSLAVSLGERATINCKSSQSLLYSSDQKNYLTWYQQKPGQPPKLLIYWASTRESGVPDRFSGSGSGTDFTLTISSLQAEDVAVYYCQQYFIYPFTFGQGTKLEIK

SEQ ID NO: 140 - protein, 113 aa, synthetic construct
DIVMTQSPDSLAVSLGERATISCKSSQSLLYSSDQKNYLTWYQQKPGQSPKLLIYWASTRESGVPDRFSGSGSGTDFTLTISSLQAEDVAVYYCQQYFIYPFTFGQGTKLEIK

SEQ ID NO: 141 - protein, 113 aa, synthetic construct
DIVMTQSPDSLAVSLGERATINCKSSQSLLYSSDQKNYLTWYQQKPGQPPKLLIYWASTRYSGVPDRFSGSGSGTDFTLTISSLQAEDVAVYYCQQYYIYPFTFGQGTKLEIK

SEQ ID NO: 142 - protein, 113 aa, synthetic construct
DIVMTQSPDSLAVSLGERATINCKSSQSLLYSSDQKNYLAWYQQKPGQPPKLLIYWASTRASGVPDRFSGSGSGTDFTLTISSLQAEDVAVYYCQQYYIYPLTFGGGTKVEIK

SEQ ID NO: 143 - protein, 113 aa, synthetic construct
DIVMTQSPASLTVSLGERVTLNCKSSQSLLYSSNQKNYLAWYQQKPGQAPKLLIYWASTRESGVPDRFSGSGSGTDFTLTISSVQAEDFAVYYCQQYYIYPLTFGQGTKLELK

SEQ ID NO: 144 - protein, 113 aa, synthetic construct
DIVMTQSPDSLAVSLGERATISCKSSQSLLYSSNQKNYLAWYQQKPGQSPKLLIYWASTRESGVPDRFSGSGSGTDFTLTISSLQAEDVAVYYCQQYYIYPLTFGGGTKVEIK

SEQ ID NO: 145 - protein, 113 aa, synthetic construct; identical to SEQ ID NO: 143

SEQ ID NO: 146 - protein, 113 aa, synthetic construct
DIVMTQSPSSLSVSVGERVTISCKSSQSLLYSSNQKNYLAWYQQKPGQAPKLLIYWASTRESGVPDRFSGSGSGTDFTLTISSVQAEDFAVYYCQQYYIYPLTFGQGTKVEIK

SEQ ID NO: 147 - protein, 113 aa, synthetic construct
DIVMTQSPDSLAVSLGERATINCKSSQSLLYSSDQKNYLTWYQQKPGQPPKLLIYWASTRESGVPDRFSGSGSGTDFTLKISRVEAEDVGVYYCQQYFIYPFTFGQGTKLEIK

SEQ ID NO: 148 - protein, 330 aa, synthetic construct
ASTKGPSVFPLAPSSKSTSGGTAALGCLVKDYFPEPVTVSWNSGALTSGVHTFPAVLQSSGLYSLSSVVTVPSSSLGTQTYICNVNHKPSNTKVDKRVEPKSCDKTHTCPPCPAPELLGGPSVFLFPPKPKDTLMISRTPEVTCVVVDVSHEDPEVKFNWYVDGVEVHNAKTKPREEQYNSTYRVVSVLTVLHQDWLNGKEYKCKVSNKALPAPIEKTISKAKGQPREPQVYTLPPSREEMTKNQVSLTCLVKGFYPSDIAVEWESNGQPENNYKTTPPVLDSDGSFFLYSKLTVDKSRWQQGNVFSCSVMHEALHNHYTQKSLSLSPGK

SEQ ID NO: 149 - protein, 326 aa, synthetic construct
ASTKGPSVFPLAPCSRSTSESTAALGCLVKDYFPEPVTVSWNSGALTSGVHTFPAVLQSSGLYSLSSVVTVPSSNFGTQTYTCNVDHKPSNTKVDKTVERKCCVECPPCPAPPVAGPSVFLFPPKPKDTLMISRTPEVTCVVVDVSHEDPEVQFNWYVDGVEVHNAKTKPREEQFNSTFRVVSVLTVVHQDWLNGKEYKCKVSNKGLPAPIEKTISKTKGQPREPQVYTLPPSREEMTKNQVSLTCLVKGFYPSDISVEWESNGQPENNYKTTPPMLDSDGSFFLYSKLTVDKSRWQQGNVFSCSVMHEALHNHYTQKSLSLSPGK

SEQ ID NO: 150 - protein, 327 aa, synthetic construct
ASTKGPSVFPLAPCSRSTSESTAALGCLVKDYFPEPVTVSWNSGALTSGVHTFPAVLQSSGLYSLSSVVTVPSSSLGTKTYTCNVDHKPSNTKVDKRVESKYGPPCPPCPAPEFLGGPSVFLFPPKPKDTLMISRTPEVTCVVVDVSQEDPEVQFNWYVDGVEVHNAKTKPREEQFNSTYRVVSVLTVLHQDWLNGKEYKCKVSNKGLPSSIEKTISKAKGQPREPQVYTLPPSQEEMTKNQVSLTCLVKGFYPSDIAVEWESNGQPENNYKTTPPVLDSDGSFFLYSRLTVDKSRWQEGNVFSCSVMHEALHNHYTQKSLSLSLGK

SEQ ID NO: 151 - protein, 107 aa, synthetic construct [sequence omitted]

SEQ ID NO: 152 - protein, 6 aa, synthetic construct
  SITE 1: note = misc_feature - X at position 1 is R, N or S
  SITE 4: note = misc_feature - X at position 4 is S or T
XGYXWH

SEQ ID NO: 153 - protein, 16 aa, synthetic construct
  SITE 1: note = misc_feature - X at position 1 is Y, V or F
  SITE 2: note = misc_feature - X at position 2 is I or T
  SITE 3: note = misc_feature - X at position 3 is H, W or Q
  SITE 4: note = misc_feature - X at position 4 is H, G, Y or F
  SITE 5: note = misc_feature - X at position 5 is R, S or D
  SITE 7: note = misc_feature - X at position 7 is S, T, N or A
  SITE 9: note = misc_feature - X at position 9 is N or K
  SITE 11: note = misc_feature - X at position 11 is N or H
  SITE 12: note = misc_feature - X at position 12 is P or S
  SITE 13: note = misc_feature - X at position 13 is S or A
  SITE 15: note = misc_feature - X at position 15 is K or I
  SITE 16: note = misc_feature - X at position 16 is S or N
XXXXXGXTXYXXXLXX

SEQ ID NO: 154 - skipped

SEQ ID NO: 155 - protein, 17 aa, synthetic construct
  SITE 1: note = misc_feature - X at position 1 is K or Q
  SITE 10: note = misc_feature - X at position 10 is N, S or K
  SITE 11: note = misc_feature - X at position 11 is N or D
  SITE 16: note = misc_feature - X at position 16 is L or S
  SITE 17: note = misc_feature - X at position 17 is A, T or V
XSSQSLLYSXXQKNYXX

SEQ ID NO: 156-157 - skipped (2 entries)